European Patent Application EP 4 465 036 A1, published November 20, 2024. Title: ANALISIS METHOD FOR NEUROGRANIN-RELATED PEPTIDE. Applicant: SHIMADZU CORPORATION. The sequence listing filed with the application follows.

SEQUENCE LISTING (3 sequences)

SEQ ID NO: 1 - protein, 33 aa, Homo sapiens
RKKIKSGERGRKGPGPGGPGGAGVARGGAGGGP

SEQ ID NO: 2 - protein, 43 aa, Homo sapiens
IQASFRGHMARKKIKSGERGRKGPGPGGPGGAGVARGGAGGGP

SEQ ID NO: 3 - protein, 29 aa, Homo sapiens
ERGRKGPGPGGPGGAGVARGGAGGGPSGD